European Patent Specification EP 3 700 918 B1, published August 27, 2025. Title: SYSTEME D'EXPRESSION BACULOVIRUS. Applicant: CENTRE NATIONAL DE LA RECHERCHE SCIENTIFIQUE (CNRS) INSTITUT NATIONAL DE LA RECHERCHE AGRONOMIQUE. The sequence listing filed with the application follows.

SEQUENCE LISTING (21 sequences)

SEQ ID NO: 1 - DNA, 75 bp, Artificial Sequence
  P10 wild
ataagaattattatcaaatcatttgtatattaattaaaatactatactgtaaattacattttatttacaatcatg

SEQ ID NO: 2 - DNA, 71 bp, Artificial Sequence
  P10S1A
ataagtattttaatcttttcgtttgtataaattaatttatactatactgtataaaaaaacctataaatatg

SEQ ID NO: 3 - DNA, 71 bp, Artificial Sequence
  P10S1B
ataagtattttaatcttttcgtttgtaccactgcagtggtactatactgtataaaaaaacctataaatatg

SEQ ID NO: 4 - DNA, 19 bp, Artificial Sequence
  Sens39k
cgcagcaattccagcgagc

SEQ ID NO: 5 - DNA, 65 bp, Artificial Sequence
  Anti-sens mut39k
ctctagacctaaggcataaaagttttttatttaatctgacatatttgtatcttgtgtattatcgc

SEQ ID NO: 6 - DNA, 57 bp, Artificial Sequence
  Sens mut39k
gccttaggtctagagtatatttaatggtttttattattgttattattaataccctcc

SEQ ID NO: 7 - DNA, 21 bp, Artificial Sequence
  Antisens 39k
cctggtaatttttgaccacgg

SEQ ID NO: 8 - DNA, 20 bp, Artificial Sequence
  Sens iap2
gatattgtgtgctcaatgtc

SEQ ID NO: 9 - DNA, 30 bp, Artificial Sequence
  Anti-sens BstBI
cctaaggtctagattcgaatacgtgtgtcg

SEQ ID NO: 10 - DNA, 37 bp, Artificial Sequence
  Sens BstBI
cgaatctagaccttaggccgcggctaagcgttaaacc

SEQ ID NO: 11 - DNA, 23 bp, Artificial Sequence
  Anti-sens iap2
cgatcaccgtcgctgtcgtcttc

SEQ ID NO: 12 - DNA, 24 bp, Artificial Sequence
  Sens orf51
ggaaaactctttccgaagacgaac

SEQ ID NO: 13 - DNA, 40 bp, Artificial Sequence
  Anti-sens Xba/orf51
cctaaggtctagagtgccttttgtttgctattttgcgccg

SEQ ID NO: 14 - DNA, 31 bp, Artificial Sequence
  Sens Xba/orf51
ctctagaccttaggtccgcgctctcccacgc

SEQ ID NO: 15 - DNA, 28 bp, Artificial Sequence
  Anti-sens orf51
ggtgcagaacataatgacgtggccttac

SEQ ID NO: 16 - DNA, 116 bp, Artificial Sequence
  gene gp37 modified
tttagccatttgagcgtatctgcattcgtcgtctagacctaggatcccgcagcaaacaatgcaattaataatgcaatgattatgattatacttatagaacactaatcggaataata

SEQ ID NO: 17 - DNA, 112 bp, Artificial sequence
  Synthetic promoter P10S1
ataagtattttaatcttttcgtttgtatattaattaaaatactatactgtataaaaaaacctataaatatcccggattattcataccgtcccaccatcgggcgtacgccacc

SEQ ID NO: 18 - DNA, 32 bp, Artificial Sequence
  PCR primer senspif1
gaatacaacgccacatctattcctagtacaac

SEQ ID NO: 19 - DNA, 50 bp, Artificial Sequence
  PCR primer pif1bac5'
ctagaggcgttaacctaaggtacttattggagaatgtccgagtatttttg

SEQ ID NO: 20 - DNA, 50 bp, Artificial Sequence
  PCR primer pif1for3'
ccttaggttaacgcctctagaacatgagcattttaaaagttgtagaagcg

SEQ ID NO: 21 - DNA, 33 bp, Artificial Sequence
  PCR primer revpif1
cattaacaattactacggcgcattttgaccatc